European Patent Application EP 4 144 745 A1, published March 8, 2023. Title: SEQUENCING METHOD, ANALYSIS METHOD THEREFOR AND ANALYSIS SYSTEM THEREOF, COMPUTER-READABLE STORAGE MEDIUM, AND ELECTRONIC DECIVE. Applicant: GENEMIND BIOSCIENCES COMPANY LIMITED. The sequence listing filed with the application follows.

SEQUENCE LISTING (4 sequences)

SEQ ID NO: 1 - DNA, 51 bp, Artificial Sequence
  misc_feature (1)..(51): primer
ctcagatcctacaacgacgctctaccgatgaagatgtgtataagagacagt

SEQ ID NO: 2 - DNA, 51 bp, Artificial Sequence
  misc_feature (1)..(51): primer
ctgtctcttatacacatctgagtggaactggatggtcgcaggtatcaagga

SEQ ID NO: 3 - DNA, 43 bp, Artificial Sequence
  misc_feature (1)..(43): primer
ctacaacgacgctctaccgatgaagatgtgtataagagacagt

SEQ ID NO: 4 - DNA, 62 bp, Artificial Sequence
  misc_feature (1)..(62): probe
tttttttttttccttgatacctgcgaccatccagttccactcagatgtgtataagagacagt